European Patent Application EP 4 151 206 A1, published March 22, 2023. Title: A pharmaceutical composition for use in treating a subject having a hypoxia condition due to  respiratory failure and the like. Applicant: TOKYO MEDICAL AND DENTAL UNIVERSITY. The sequence listing filed with the application follows.

SEQUENCE LISTING (8 sequences)

SEQ ID NO: 1 - DNA, 20 bp, Artificial Sequence
  Vegfa-F
aggctgctgtaacgatgaag

SEQ ID NO: 2 - DNA, 20 bp, Artificial Sequence
  Vegfa-R
tctcctatgtgctggctttg

SEQ ID NO: 3 - DNA, 20 bp, Artificial Sequence
  Anxa1-F
ccagcactccagctttcttt

SEQ ID NO: 4 - DNA, 20 bp, Artificial Sequence
  Anxa1-R
tccgaacgggagaccataat

SEQ ID NO: 5 - DNA, 22 bp, Artificial Sequence
  Spon1-F
agagaaccaggagggagataag

SEQ ID NO: 6 - DNA, 23 bp, Artificial Sequence
  Spon1-R
gccacaggacagttactcataaa

SEQ ID NO: 7 - DNA, 21 bp, Artificial Sequence
  Glud1-F
taccgtttggaggtgctaaag

SEQ ID NO: 8 - DNA, 22 bp, Artificial Sequence
  Glud1-R
ccatagtgaacctccgtgtaat